European Patent Application EP 4 471 151 A1, published December 4, 2024. Title: VIRAL VECTOR AND APPLICATION THEREOF. Applicant: SUNSHINE LAKE PHARMA CO., LTD. The sequence listing filed with the application follows.

SEQUENCE LISTING (56 sequences)

SEQ ID NO: 1 - protein, 495 aa, synthetic construct
KFTIVFPHNQKGNWKNVPSNYHYCPSSSDLNWHNDLIGTALQVKMPKSHKAIQADGWMCHASKWVTTCDFRWYGPKYITHSIRSFTPSVEQCKESIEQTKQGTWLNPGFPPQSCGYATVTDAEAVIVQVTPHHVLVDEYTGEWVDSQFINGKCSNYICPTVHNSTTWHSDYKVKGLCDSNLISMDITFFSEDGELSSLGKEGTGFRSNYFAYETGGKACKMQYCKHWGVRLPSGVWFEMADKDLFAAARFPECPEGSSISAPSQTSVDVSLIQDVERILDYSLCQETWSKIRAGLPISPVDLSYLAPKNPGTGPAFTIINGTLKYFETRYIRVDIAAPILSRMVGMISGTTTERELWDDWAPYEDVEIGPNGVLRTSSGYKFPLYMIGHGMLDSDLHLSSKAQVFEHPHIQDAASQLPDDESLFFGDTGLSKNPIELVEGWFSSWKSSIASFFFIIGLIIGLFLVLRVGIHLCIKLKHTKKRQIYTDIEMNRLGK

SEQ ID NO: 2 - protein, 495 aa, synthetic construct
KFTIVFPHNQKGNWKNVPSNYHYCPSSSDLNWHNDLIGTALQVKMPQSHKAIQADGWMCHASKWVTTCDFRWYGPKYITHSIRSFTPSVEQCKESIEQTKQGTWLNPGFPPQSCGYATVTDAEAVIVQVTPHHVLVDEYTGEWVDSQFINGKCSNYICPTVHNSTTWHSDYKVKGLCDSNLISMDITFFSEDGELSSLGKEGTGFRSNYFAYETGGKACKMQYCKHWGVRLPSGVWFEMADKDLFAAARFPECPEGSSISAPSQTSVDVSLIQDVERILDYSLCQETWSKIRAGLPISPVDLSYLAPKNPGTGPAFTIINGTLKYFETRYIRVDIAAPILSRMVGMISGTTTEQELWDDWAPYEDVEIGPNGVLRTSSGYKFPLYMIGHGMLDSDLHLSSKAQVFEHPHIQDAASQLPDDESLFFGDTGLSKNPIELVEGWFSSWKSSIASFFFIIGLIIGLFLVLRVGIHLCIKLKHTKKRQIYTDIEMNRLGK

SEQ ID NO: 3 - protein, 243 aa, synthetic construct
QVQLVQSGAEVKKPGASVKVSCKASGYTFTSYYIHWVRQAPGQGLEWIGCIYPGNVNTNYNEKFKDRATLTVDTSISTAYMELSRLRSDDTAVYFCTRSHYGLDWNFDVWGQGTTVTVSSGGGGSGGGGSGGGGSDIQMTQSPSSLSASVGDRVTITCHASQNIYVWLNWYQQKPGKAPKLLIYKASNLHTGVPSRFSGSGSGTDFTLTISSLQPEDFATYYCQQGQTYPYTFGGGTKVEIKE

SEQ ID NO: 4 - protein, 247 aa, synthetic construct
DIELTQSPASLAVSLGQRATISCRASESVEYYVTSLMQWYQQKPGQPPKLLIFAASNVESGVPARFSGSGSGTNFSLNIHPVDEDDVAMYFCQQSRKVPYTFGGGTKLEIKRGGGGSGGGGSGGGGSQVQLQESGPGLVTPSQSLSITCTVSGFSLSDYGVHWVRQSPGQGLEWLGVIWAGGGTNYNSALMSRKSISKDNSKSQVFLKMNSLQADDTAVYYCARDKGYSYYYSMDYWGQGTTVTVSS

SEQ ID NO: 5 - protein, 243 aa, synthetic construct
DIKLQQSGAELARPGASVKMSCKTSGYTFTRYTMHWVKQRPGQGLEWIGYINPSRGYTNYNQKFKDKATLTTDKSSSTAYMQLSSLTSEDSAVYYCARYYDDHYCLDYWGQGTTLTVSSVEGGSGGSGGSGGSGGVDDIQLTQSPAIMSASPGEKVTMTCRASSSVSYMNWYQQKSGTSPKRWIYDTSKVASGVPYRFSGSGSGTSYSLTISSMEAEDAATYYCQQWSSNPLTFGAGTKLELK

SEQ ID NO: 6 - protein, 241 aa, synthetic construct
QVQLQQSGAELARPGASVKMSCKASGYTFTRYTMHWVKQRPGQGLEWIGYINPSRGYTNYNQKFKDKATLTTDKSSSTAYMQLSSLTSEDSAVYYCARYYDDHYCLDYWGQGTTLTVSSGGGGSGGGGSGGGGSQIVLTQSPAIMSASPGEKVTMTCSASSSVSYMNWYQQKSGTSPKRWIYDTSKLASGVPAHFRGSGSGTSYSLTISGMEAEDAATYYCQQWSSNPFTFGSGTKLEINR

SEQ ID NO: 7 - protein, 25 aa, synthetic construct
GGGGSGGGGSGGGGSGGGGSGGGGS

SEQ ID NO: 8 - protein, 20 aa, synthetic construct
GGGGSGGGGSGGGGSGGGGS

SEQ ID NO: 9 - protein, 15 aa, synthetic construct
GGGGSGGGGSGGGGS

SEQ ID NO: 10 - protein, 16 aa, synthetic construct
EAAAKEAAAKEAAAKE

SEQ ID NO: 11 - protein, 20 aa, synthetic construct
EAAAKEAAAKEAAAKEAAAK

SEQ ID NO: 12 - protein, 6 aa, synthetic construct
AAATTT

SEQ ID NO: 13 - protein, 91 aa, synthetic construct
FEHPHIQDAASQLPDDESLFFGDTGLSKNPIELVEGWFSSWKSSIASFFFIIGLIIGLFLVLRVGIHLCIKLKHTKKRQIYTDIEMNRLGK

SEQ ID NO: 14 - protein, 340 aa, synthetic construct
QVQLVQSGAEVKKPGASVKVSCKASGYTFTSYYIHWVRQAPGQGLEWIGCIYPGNVNTNYNEKFKDRATLTVDTSISTAYMELSRLRSDDTAVYFCTRSHYGLDWNFDVWGQGTTVTVSSGGGGSGGGGSGGGGSDIQMTQSPSSLSASVGDRVTITCHASQNIYVWLNWYQQKPGKAPKLLIYKASNLHTGVPSRFSGSGSGTDFTLTISSLQPEDFATYYCQQGQTYPYTFGGGTKVEIKEAAATTTFEHPHIQDAASQLPDDESLFFGDTGLSKNPIELVEGWFSSWKSSIASFFFIIGLIIGLFLVLRVGIHLCIKLKHTKKRQIYTDIEMNRLGK

SEQ ID NO: 15 - protein, 340 aa, synthetic construct
DIKLQQSGAELARPGASVKMSCKTSGYTFTRYTMHWVKQRPGQGLEWIGYINPSRGYTNYNQKFKDKATLTTDKSSSTAYMQLSSLTSEDSAVYYCARYYDDHYCLDYWGQGTTLTVSSVEGGSGGSGGSGGSGGVDDIQLTQSPAIMSASPGEKVTMTCRASSSVSYMNWYQQKSGTSPKRWIYDTSKVASGVPYRFSGSGSGTSYSLTISSMEAEDAATYYCQQWSSNPLTFGAGTKLELKAAATTTFEHPHIQDAASQLPDDESLFFGDTGLSKNPIELVEGWFSSWKSSIASFFFIIGLIIGLFLVLRVGIHLCIKLKHTKKRQIYTDIEMNRLGK

SEQ ID NO: 16 - protein, 608 aa, synthetic construct
QVQLVQSGAEVKKPGASVKVSCKASGYTFTSYYIHWVRQAPGQGLEWIGCIYPGNVNTNYNEKFKDRATLTVDTSISTAYMELSRLRSDDTAVYFCTRSHYGLDWNFDVWGQGTTVTVSSGGGGSGGGGSGGGGSDIQMTQSPSSLSASVGDRVTITCHASQNIYVWLNWYQQKPGKAPKLLIYKASNLHTGVPSRFSGSGSGTDFTLTISSLQPEDFATYYCQQGQTYPYTFGGGTKVEIKEGGGGSGGGGSGGGGSGGGGSGGGGSDIKLQQSGAELARPGASVKMSCKTSGYTFTRYTMHWVKQRPGQGLEWIGYINPSRGYTNYNQKFKDKATLTTDKSSSTAYMQLSSLTSEDSAVYYCARYYDDHYCLDYWGQGTTLTVSSVEGGSGGSGGSGGSGGVDDIQLTQSPAIMSASPGEKVTMTCRASSSVSYMNWYQQKSGTSPKRWIYDTSKVASGVPYRFSGSGSGTSYSLTISSMEAEDAATYYCQQWSSNPLTFGAGTKLELKAAATTTFEHPHIQDAASQLPDDESLFFGDTGLSKNPIELVEGWFSSWKSSIASFFFIIGLIIGLFLVLRVGIHLCIKLKHTKKRQIYTDIEMNRLGK

SEQ ID NO: 17 - protein, 608 aa, synthetic construct
DIKLQQSGAELARPGASVKMSCKTSGYTFTRYTMHWVKQRPGQGLEWIGYINPSRGYTNYNQKFKDKATLTTDKSSSTAYMQLSSLTSEDSAVYYCARYYDDHYCLDYWGQGTTLTVSSVEGGSGGSGGSGGSGGVDDIQLTQSPAIMSASPGEKVTMTCRASSSVSYMNWYQQKSGTSPKRWIYDTSKVASGVPYRFSGSGSGTSYSLTISSMEAEDAATYYCQQWSSNPLTFGAGTKLELKGGGGSGGGGSGGGGSGGGGSGGGGSQVQLVQSGAEVKKPGASVKVSCKASGYTFTSYYIHWVRQAPGQGLEWIGCIYPGNVNTNYNEKFKDRATLTVDTSISTAYMELSRLRSDDTAVYFCTRSHYGLDWNFDVWGQGTTVTVSSGGGGSGGGGSGGGGSDIQMTQSPSSLSASVGDRVTITCHASQNIYVWLNWYQQKPGKAPKLLIYKASNLHTGVPSRFSGSGSGTDFTLTISSLQPEDFATYYCQQGQTYPYTFGGGTKVEIKEAAATTTFEHPHIQDAASQLPDDESLFFGDTGLSKNPIELVEGWFSSWKSSIASFFFIIGLIIGLFLVLRVGIHLCIKLKHTKKRQIYTDIEMNRLGK

SEQ ID NO: 18 - protein, 344 aa, synthetic construct
DIELTQSPASLAVSLGQRATISCRASESVEYYVTSLMQWYQQKPGQPPKLLIFAASNVESGVPARFSGSGSGTNFSLNIHPVDEDDVAMYFCQQSRKVPYTFGGGTKLEIKRGGGGSGGGGSGGGGSQVQLQESGPGLVTPSQSLSITCTVSGFSLSDYGVHWVRQSPGQGLEWLGVIWAGGGTNYNSALMSRKSISKDNSKSQVFLKMNSLQADDTAVYYCARDKGYSYYYSMDYWGQGTTVTVSSAAATTTFEHPHIQDAASQLPDDESLFFGDTGLSKNPIELVEGWFSSWKSSIASFFFIIGLIIGLFLVLRVGIHLCIKLKHTKKRQIYTDIEMNRLGK

SEQ ID NO: 19 - protein, 338 aa, synthetic construct
QVQLQQSGAELARPGASVKMSCKASGYTFTRYTMHWVKQRPGQGLEWIGYINPSRGYTNYNQKFKDKATLTTDKSSSTAYMQLSSLTSEDSAVYYCARYYDDHYCLDYWGQGTTLTVSSGGGGSGGGGSGGGGSQIVLTQSPAIMSASPGEKVTMTCSASSSVSYMNWYQQKSGTSPKRWIYDTSKLASGVPAHFRGSGSGTSYSLTISGMEAEDAATYYCQQWSSNPFTFGSGTKLEINRAAATTTFEHPHIQDAASQLPDDESLFFGDTGLSKNPIELVEGWFSSWKSSIASFFFIIGLIIGLFLVLRVGIHLCIKLKHTKKRQIYTDIEMNRLGK

SEQ ID NO: 20 - protein, 610 aa, synthetic construct
DIELTQSPASLAVSLGQRATISCRASESVEYYVTSLMQWYQQKPGQPPKLLIFAASNVESGVPARFSGSGSGTNFSLNIHPVDEDDVAMYFCQQSRKVPYTFGGGTKLEIKRGGGGSGGGGSGGGGSQVQLQESGPGLVTPSQSLSITCTVSGFSLSDYGVHWVRQSPGQGLEWLGVIWAGGGTNYNSALMSRKSISKDNSKSQVFLKMNSLQADDTAVYYCARDKGYSYYYSMDYWGQGTTVTVSSGGGGSGGGGSGGGGSGGGGSGGGGSQVQLQQSGAELARPGASVKMSCKASGYTFTRYTMHWVKQRPGQGLEWIGYINPSRGYTNYNQKFKDKATLTTDKSSSTAYMQLSSLTSEDSAVYYCARYYDDHYCLDYWGQGTTLTVSSGGGGSGGGGSGGGGSQIVLTQSPAIMSASPGEKVTMTCSASSSVSYMNWYQQKSGTSPKRWIYDTSKLASGVPAHFRGSGSGTSYSLTISGMEAEDAATYYCQQWSSNPFTFGSGTKLEINRAAATTTFEHPHIQDAASQLPDDESLFFGDTGLSKNPIELVEGWFSSWKSSIASFFFIIGLIIGLFLVLRVGIHLCIKLKHTKKRQIYTDIEMNRLGK

SEQ ID NO: 21 - DNA, 1533 bp, synthetic construct
  source 1..1533: mol_type = other DNA
atgaagtgccttttgtacttagcctttttattcattggggtgaattgcaagttcaccatagtttttccacacaaccaaaaaggaaactggaaaaatgttccttctaattaccattattgcccgtcaagctcagatttaaattggcataatgacttaataggcacagccttacaagtcaaaatgccccaaagtcacaaggctattcaagcagacggttggatgtgtcatgcttccaaatgggtcactacttgtgatttccgctggtatggaccgaagtatataacacattccatccgatccttcactccatctgtagaacaatgcaaggaaagcattgaacaaacgaaacaaggaacttggctgaatccaggcttccctcctcaaagttgtggatatgcaactgtgacggatgccgaagcagtgattgtccaggtgactcctcaccatgtgctggttgatgaatacacaggagaatgggttgattcacagttcatcaacggaaaatgcagcaattacatatgccccactgtccataactctacaacctggcattctgactataaggtcaaagggctatgtgattctaacctcatttccatggacatcaccttcttctcagaggacggagagctatcatccctgggaaaggagggcacagggttcagaagtaactactttgcttatgaaactggaggcaaggcctgcaaaatgcaatactgcaagcattggggagtcagactcccatcaggtgtctggttcgagatggctgataaggatctctttgctgcagccagattccctgaatgcccagaagggtcaagtatctctgctccatctcagacctcagtggatgtaagtctaattcaggacgttgagaggatcttggattattccctctgccaagaaacctggagcaaaatcagagcgggtcttccaatctctccagtggatctcagctatcttgctcctaaaaacccaggaaccggtcctgctttcaccataatcaatggtaccctaaaatactttgagaccagatacatcagagtcgatattgctgctccaatcctctcaagaatggtcggaatgatcagtggaactaccacagaacaggaactgtgggatgactgggcaccatatgaagacgtggaaattggacccaatggagttctgaggaccagttcaggatataagtttcctttatacatgattggacatggtatgttggactccgatcttcatcttagctcaaaggctcaggtgttcgaacatcctcacattcaagacgctgcttcgcaacttcctgatgatgagagtttattttttggtgatactgggctatccaaaaatccaatcgagcttgtagaaggttggttcagtagttggaaaagctctattgcctcttttttctttatcatagggttaatcattggactattcttggttctccgagttggtatccatctttgcattaaattaaagcacaccaagaaaagacagatttatacagacatagagatgaaccgacttggaaag

SEQ ID NO: 22 - DNA, 1020 bp, synthetic construct
  source 1..1020: mol_type = other DNA
caggtgcagctggtgcagtctggggctgaggtgaagaagcctggggcctcagtgaaggtctcctgcaaggcttctggatacaccttcaccagctactatatacactgggtgcgacaggcccctggacaagggcttgagtggattggatgtatttatcctggaaatgtcaatactaactataatgagaagttcaaggacagggccaccctgaccgtagacacgtccatcagcacagcctacatggagctgagcaggctgagatctgacgacacggccgtgtatttctgtacaagatcacactacggcctcgactggaacttcgatgtctggggccaagggaccacggtcaccgtctcctcaggtggaggcggttcaggcggaggtggcagcggcggtggcgggtcggacatccagatgacccagtctccatcctccctgtctgcatctgtaggagacagagtcaccatcacttgccatgccagtcaaaacatttatgtttggttaaactggtatcagcagaaaccagggaaagcccctaagctcctgatctataaggcttccaacctgcacacaggggtcccatcaaggttcagtggcagtggatctgggacagatttcactctcaccatcagcagtctgcaacctgaagattttgcaacttactactgtcaacagggtcaaacttatccgtacacgttcggcggagggaccaaggtggagatcaaagaggcggccgcaactaccaccttcgaacatcctcacattcaagacgctgcttcgcaacttcctgatgatgagagtttattttttggtgatactgggctatccaaaaatccaatcgagcttgtagaaggttggttcagtagttggaaaagctctattgcctcttttttctttatcatagggttaatcattggactattcttggttctccgagttggtatccatctttgcattaaattaaagcacaccaagaaaagacagatttatacagacatagagatgaaccgacttggaaag

SEQ ID NO: 23 - DNA, 1020 bp, synthetic construct
  source 1..1020: mol_type = other DNA
gatatcaaactgcagcagtcaggggctgaactggcaagacctggggcctcagtgaagatgtcctgcaagacttctggctacacctttactaggtacacgatgcactgggtaaaacagaggcctggacagggtctggaatggattggatacattaatcctagccgtggttatactaattacaatcagaagttcaaggacaaggccacattgactacagacaaatcctccagcacagcctacatgcaactgagcagcctgacatctgaggactctgcagtctattactgtgcaagatattatgatgatcattactgccttgactactggggccaaggcaccactctcacagtctcctcagtcgaaggtggaagtggaggttctggtggaagtggaggttcaggtggagtcgacgacattcagctgacccagtctccagcaatcatgtctgcatctccaggggagaaggtcaccatgacctgcagagccagttcaagtgtaagttacatgaactggtaccagcagaagtcaggcacctcccccaaaagatggatttatgacacatccaaagtggcttctggagtcccttatcgcttcagtggcagtgggtctgggacctcatactctctcacaatcagcagcatggaggctgaagatgctgccacttattactgccaacagtggagtagtaacccgctcacgttcggtgctgggaccaagctggagctgaaagcggccgcaactaccaccttcgaacatcctcacattcaagacgctgcttcgcaacttcctgatgatgagagtttattttttggtgatactgggctatccaaaaatccaatcgagcttgtagaaggttggttcagtagttggaaaagctctattgcctcttttttctttatcatagggttaatcattggactattcttggttctccgagttggtatccatctttgcattaaattaaagcacaccaagaaaagacagatttatacagacatagagatgaaccgacttggaaag

SEQ ID NO: 24 - DNA, 1824 bp, synthetic construct
  source 1..1824: mol_type = other DNA
caggtgcagctggtgcagtctggggctgaggtgaagaagcctggggcctcagtgaaggtctcctgcaaggcttctggatacaccttcaccagctactatatacactgggtgcgacaggcccctggacaagggcttgagtggattggatgtatttatcctggaaatgtcaatactaactataatgagaagttcaaggacagggccaccctgaccgtagacacgtccatcagcacagcctacatggagctgagcaggctgagatctgacgacacggccgtgtatttctgtacaagatcacactacggcctcgactggaacttcgatgtctggggccaagggaccacggtcaccgtctcctcaggtggaggcggttcaggcggaggtggcagcggcggtggcgggtcggacatccagatgacccagtctccatcctccctgtctgcatctgtaggagacagagtcaccatcacttgccatgccagtcaaaacatttatgtttggttaaactggtatcagcagaaaccagggaaagcccctaagctcctgatctataaggcttccaacctgcacacaggggtcccatcaaggttcagtggcagtggatctgggacagatttcactctcaccatcagcagtctgcaacctgaagattttgcaacttactactgtcaacagggtcaaacttatccgtacacgttcggcggagggaccaaggtggagatcaaagagggaggcggcggcagcggcgggggagggtccggagggggtggttctggtggaggaggatcgggaggcggtggcagcgatatcaaactgcagcagtcaggggctgaactggcaagacctggggcctcagtgaagatgtcctgcaagacttctggctacacctttactaggtacacgatgcactgggtaaaacagaggcctggacagggtctggaatggattggatacattaatcctagccgtggttatactaattacaatcagaagttcaaggacaaggccacattgactacagacaaatcctccagcacagcctacatgcaactgagcagcctgacatctgaggactctgcagtctattactgtgcaagatattatgatgatcattactgccttgactactggggccaaggcaccactctcacagtctcctcagtcgaaggtggaagtggaggttctggtggaagtggaggttcaggtggagtcgacgacattcagctgacccagtctccagcaatcatgtctgcatctccaggggagaaggtcaccatgacctgcagagccagttcaagtgtaagttacatgaactggtaccagcagaagtcaggcacctcccccaaaagatggatttatgacacatccaaagtggcttctggagtcccttatcgcttcagtggcagtgggtctgggacctcatactctctcacaatcagcagcatggaggctgaagatgctgccacttattactgccaacagtggagtagtaacccgctcacgttcggtgctgggaccaagctggagctgaaagcggccgcaactaccaccttcgaacatcctcacattcaagacgctgcttcgcaacttcctgatgatgagagtttattttttggtgatactgggctatccaaaaatccaatcgagcttgtagaaggttggttcagtagttggaaaagctctattgcctcttttttctttatcatagggttaatcattggactattcttggttctccgagttggtatccatctttgcattaaattaaagcacaccaagaaaagacagatttatacagacatagagatgaaccgacttggaaag

SEQ ID NO: 25 - DNA, 1824 bp, synthetic construct
  source 1..1824: mol_type = other DNA
gatatcaaactgcagcagtcaggggctgaactggcaagacctggggcctcagtgaagatgtcctgcaagacttctggctacacctttactaggtacacgatgcactgggtaaaacagaggcctggacagggtctggaatggattggatacattaatcctagccgtggttatactaattacaatcagaagttcaaggacaaggccacattgactacagacaaatcctccagcacagcctacatgcaactgagcagcctgacatctgaggactctgcagtctattactgtgcaagatattatgatgatcattactgccttgactactggggccaaggcaccactctcacagtctcctcagtcgaaggtggaagtggaggttctggtggaagtggaggttcaggtggagtcgacgacattcagctgacccagtctccagcaatcatgtctgcatctccaggggagaaggtcaccatgacctgcagagccagttcaagtgtaagttacatgaactggtaccagcagaagtcaggcacctcccccaaaagatggatttatgacacatccaaagtggcttctggagtcccttatcgcttcagtggcagtgggtctgggacctcatactctctcacaatcagcagcatggaggctgaagatgctgccacttattactgccaacagtggagtagtaacccgctcacgttcggtgctgggaccaagctggagctgaaaggaggcggcggcagcggcgggggagggtccggagggggtggttctggtggaggaggatcgggaggcggtggcagccaggtgcagctggtgcagtctggggctgaggtgaagaagcctggggcctcagtgaaggtctcctgcaaggcttctggatacaccttcaccagctactatatacactgggtgcgacaggcccctggacaagggcttgagtggattggatgtatttatcctggaaatgtcaatactaactataatgagaagttcaaggacagggccaccctgaccgtagacacgtccatcagcacagcctacatggagctgagcaggctgagatctgacgacacggccgtgtatttctgtacaagatcacactacggcctcgactggaacttcgatgtctggggccaagggaccacggtcaccgtctcctcaggtggaggcggttcaggcggaggtggcagcggcggtggcgggtcggacatccagatgacccagtctccatcctccctgtctgcatctgtaggagacagagtcaccatcacttgccatgccagtcaaaacatttatgtttggttaaactggtatcagcagaaaccagggaaagcccctaagctcctgatctataaggcttccaacctgcacacaggggtcccatcaaggttcagtggcagtggatctgggacagatttcactctcaccatcagcagtctgcaacctgaagattttgcaacttactactgtcaacagggtcaaacttatccgtacacgttcggcggagggaccaaggtggagatcaaagaggcggccgcaactaccaccttcgaacatcctcacattcaagacgctgcttcgcaacttcctgatgatgagagtttattttttggtgatactgggctatccaaaaatccaatcgagcttgtagaaggttggttcagtagttggaaaagctctattgcctcttttttctttatcatagggttaatcattggactattcttggttctccgagttggtatccatctttgcattaaattaaagcacaccaagaaaagacagatttatacagacatagagatgaaccgacttggaaag

SEQ ID NO: 26 - DNA, 48 bp, synthetic construct
  source 1..48: mol_type = other DNA
atgaagtgccttttgtacttagcctttttattcattggggtgaattgc

SEQ ID NO: 27 - protein, 16 aa, synthetic construct
MKCLLYLAFLFIGVNC

SEQ ID NO: 28 - DNA, 1494 bp, synthetic construct
  source 1..1494: mol_type = other DNA
gacatccagatgacacagactacatcctccctgtctgcctctctgggagacagagtcaccatcagttgcagggcaagtcaggacattagtaaatatttaaattggtatcagcagaaaccagatggaactgttaaactcctgatctaccatacatcaagattacactcaggagtcccatcaaggttcagtggcagtgggtctggaacagattattctctcaccattagcaacctggagcaagaagatattgccacttacttttgccaacagggtaatacgcttccgtacacgttcggaggggggaccaagctggagatcacaggtggcggtggctcgggcggtggtgggtcgggtggcggcggatctgaggtgaaactgcaggagtcaggacctggcctggtggcgccctcacagagcctgtccgtcacatgcactgtctcaggggtctcattacccgactatggtgtaagctggattcgccagcctccacgaaagggtctggagtggctgggagtaatatggggtagtgaaaccacatactataattcagctctcaaatccagactgaccatcatcaaggacaactccaagagccaagttttcttaaaaatgaacagtctgcaaactgatgacacagccatttactactgtgccaaacattattactacggtggtagctatgctatggactactggggccaaggaacctcagtcaccgtctcctcagaattcaccacgacgccagcgccgcgaccaccaacaccggcgcccaccatcgcgtcgcagcccctgtccctgcgcccagaggcgtgccggccagcggcggggggcgcagtgcacacgagggggctggacttcgcctgtgatatctacatctgggcgcccttggccgggacttgtggggtccttctcctgtcactggttatcaccctttactgcaagcgcggccgcaagaagctgctgtacatcttcaagcagcccttcatgcgccccgtgcagaccacccaggaggaggacggctgtagctgccgcttccccgaggaggaggagggcggctgcgagctgcggcgcgaccagcgcctgccccccgacgcccacaagccccccggcggcggcagcttccgcacccccatccaggaggagcaggccgacgcccacagcaccctggccaagatccgcgtgaaatttagccgcagcgccgacgcccccgcctaccagcagggccagaaccagctgtacaacgagctgaacctgggccgccgcgaggagtacgacgtgctggacaagcgccggggccgcgaccccgagatgggcggcaagccccagcgccgcaagaacccccaggagggcctgtacaacgagctgcagaaggacaagatggccgaagcctacagcgagatcggcatgaagggcgagcgccgccggggcaagggccacgacggcctgtaccagggcctgagcaccgccaccaaggacacctacgacgccctgcac

SEQ ID NO: 29 - protein, 498 aa, synthetic construct
DIQMTQTTSSLSASLGDRVTISCRASQDISKYLNWYQQKPDGTVKLLIYHTSRLHSGVPSRFSGSGSGTDYSLTISNLEQEDIATYFCQQGNTLPYTFGGGTKLEITGGGGSGGGGSGGGGSEVKLQESGPGLVAPSQSLSVTCTVSGVSLPDYGVSWIRQPPRKGLEWLGVIWGSETTYYNSALKSRLTIIKDNSKSQVFLKMNSLQTDDTAIYYCAKHYYYGGSYAMDYWGQGTSVTVSSEFTTTPAPRPPTPAPTIASQPLSLRPEACRPAAGGAVHTRGLDFACDIYIWAPLAGTCGVLLLSLVITLYCKRGRKKLLYIFKQPFMRPVQTTQEEDGCSCRFPEEEEGGCELRRDQRLPPDAHKPPGGGSFRTPIQEEQADAHSTLAKIRVKFSRSADAPAYQQGQNQLYNELNLGRREEYDVLDKRRGRDPEMGGKPQRRKNPQEGLYNELQKDKMAEAYSEIGMKGERRRGKGHDGLYQGLSTATKDTYDALH

SEQ ID NO: 30 - DNA, 1518 bp, synthetic construct
  source 1..1518: mol_type = other DNA
gacatccagatgacacagactacatcctccctgtctgcctctctgggagacagagtcaccatcagttgcagggcaagtcaggacattagtaaatatttaaattggtatcagcagaaaccagatggaactgttaaactcctgatctaccatacatcaagattacactcaggagtcccatcaaggttcagtggcagtgggtctggaacagattattctctcaccattagcaacctggagcaagaagatattgccacttacttttgccaacagggtaatacgcttccgtacacgttcggaggggggaccaagctggagatcacaggtggcggtggctcgggcggtggtgggtcgggtggcggcggatctgaggtgaaactgcaggagtcaggacctggcctggtggcgccctcacagagcctgtccgtcacatgcactgtctcaggggtctcattacccgactatggtgtaagctggattcgccagcctccacgaaagggtctggagtggctgggagtaatatggggtagtgaaaccacatactataattcagctctcaaatccagactgaccatcatcaaggacaactccaagagccaagttttcttaaaaatgaacagtctgcaaactgatgacacagccatttactactgtgccaaacattattactacggtggtagctatgctatggactactggggccaaggaacctcagtcaccgtctcctcagaattcaccacgacgccagcgccgcgaccaccaacaccggcgcccaccatcgcgtcgcagcccctgtccctgcgcccagaggcgtgccggccagcggcggggggcgcagtgcacacgagggggctggacttcgcctgtgatatctacatctgggcgcccttggccgggacttgtggggtccttctcctgtcactggttatcaccctttactgctgttggcttacaaaaaagaagtattcatccagtgtgcacgaccctaacggtgaatacatgttcatgagagcagtgaacacagccaaaaaatctagactcacagatgtgaccctaaagcgcggccgcaagaagctgctgtacatcttcaagcagcccttcatgcgccccgtgcagaccacccaggaggaggacggctgtagctgccgcttccccgaggaggaggagggcggctgcgagctgcgcgtgaaatttagccgcagcgccgacgcccccgcctaccagcagggccagaaccagctgtacaacgagctgaacctgggccgccgcgaggagtacgacgtgctggacaagcgccggggccgcgaccccgagatgggcggcaagccccagcgccgcaagaacccccaggagggcctgtacaacgagctgcagaaggacaagatggccgaagcctacagcgagatcggcatgaagggcgagcgccgccggggcaagggccacgacggcctgtaccagggcctgagcaccgccaccaaggacacctacgacgccctgcacatgcaggccctgcccccccgc

SEQ ID NO: 31 - protein, 506 aa, synthetic construct
DIQMTQTTSSLSASLGDRVTISCRASQDISKYLNWYQQKPDGTVKLLIYHTSRLHSGVPSRFSGSGSGTDYSLTISNLEQEDIATYFCQQGNTLPYTFGGGTKLEITGGGGSGGGGSGGGGSEVKLQESGPGLVAPSQSLSVTCTVSGVSLPDYGVSWIRQPPRKGLEWLGVIWGSETTYYNSALKSRLTIIKDNSKSQVFLKMNSLQTDDTAIYYCAKHYYYGGSYAMDYWGQGTSVTVSSEFTTTPAPRPPTPAPTIASQPLSLRPEACRPAAGGAVHTRGLDFACDIYIWAPLAGTCGVLLLSLVITLYCCWLTKKKYSSSVHDPNGEYMFMRAVNTAKKSRLTDVTLKRGRKKLLYIFKQPFMRPVQTTQEEDGCSCRFPEEEEGGCELRVKFSRSADAPAYQQGQNQLYNELNLGRREEYDVLDKRRGRDPEMGGKPQRRKNPQEGLYNELQKDKMAEAYSEIGMKGERRRGKGHDGLYQGLSTATKDTYDALHMQALPPR

SEQ ID NO: 32 - DNA, 1032 bp, synthetic construct
  source 1..1032: mol_type = other DNA
gacatcgagctcactcagtctccagcttctttggctgtgtctctagggcagagagccaccatctcctgcagagccagtgagagtgttgaatattatgtcacaagtttaatgcagtggtaccagcagaagccaggacagccacccaaactcctcatctttgctgcatccaacgtagaatctggggtccctgccaggtttagtggcagtgggtctgggacaaacttcagcctcaacatccatcctgtggacgaggatgatgttgcaatgtatttctgtcagcaaagtaggaaggttccttacacgttcggaggggggaccaagctggaaataaaacgagggggcggaggatccggtggaggcggaagcgggggtggaggatcccaggtgcagctgcaggagtcaggacctggcctggtgacgccctcacagagcctgtccatcacttgtactgtctctgggttttcattaagcgactatggtgttcattgggttcgccagtctccaggacagggactggagtggctgggagtaatatgggctggtggaggcacgaattataattcggctctcatgtccagaaagagcatcagcaaagacaactccaagagccaagttttcttaaaaatgaacagtctgcaagctgatgacacagccgtgtattactgtgccagagataagggatactcctattactattctatggactactggggccaaggcaccacggtcaccgtctcctcagcggccgcaactaccaccttcgaacatcctcacattcaagacgctgcttcgcaacttcctgatgatgagagtttattttttggtgatactgggctatccaaaaatccaatcgagcttgtagaaggttggttcagtagttggaaaagctctattgcctcttttttctttatcatagggttaatcattggactattcttggttctccgagttggtatccatctttgcattaaattaaagcacaccaagaaaagacagatttatacagacatagagatgaaccgacttggaaag

SEQ ID NO: 33 - DNA, 1014 bp, synthetic construct
  source 1..1014: mol_type = other DNA
caggtccagctgcagcagtctggggctgaactggcaagacctggggcctcagtgaagatgtcctgcaaggcttctggctacacctttactaggtacacgatgcactgggtaaaacagaggcctggacagggtctggaatggattggatacattaatcctagccgtggttatactaattacaatcagaagttcaaggacaaggccacattgactacagacaaatcctccagcacagcctacatgcaactgagcagcctgacatctgaggactctgcagtctattactgtgcaagatattatgatgatcattactgccttgactactggggccaaggcaccactctcacagtctcctcaggtggcggtggctccggcggtggtgggtcgggtggcggcggatctcagattgtgttgacccagtctccagcaatcatgtctgcatctccaggggagaaggttaccatgacctgcagtgccagctcaagtgtaagttacatgaactggtaccagcagaagtcaggcacctcccccaaaagatggatttatgacacatccaaactggcttctggagtccctgctcacttcaggggcagtgggtctgggacctcttactctctcacaatcagcggcatggaggctgaagatgctgccacttattactgccagcagtggagtagtaacccattcacgttcggctcggggaccaagctggagatcaaccgtgcggccgcaactaccaccttcgaacatcctcacattcaagacgctgcttcgcaacttcctgatgatgagagtttattttttggtgatactgggctatccaaaaatccaatcgagcttgtagaaggttggttcagtagttggaaaagctctattgcctcttttttctttatcatagggttaatcattggactattcttggttctccgagttggtatccatctttgcattaaattaaagcacaccaagaaaagacagatttatacagacatagagatgaaccgacttggaaag

SEQ ID NO: 34 - DNA, 1830 bp, synthetic construct
  source 1..1830: mol_type = other DNA
gacatcgagctcactcagtctccagcttctttggctgtgtctctagggcagagagccaccatctcctgcagagccagtgagagtgttgaatattatgtcacaagtttaatgcagtggtaccagcagaagccaggacagccacccaaactcctcatctttgctgcatccaacgtagaatctggggtccctgccaggtttagtggcagtgggtctgggacaaacttcagcctcaacatccatcctgtggacgaggatgatgttgcaatgtatttctgtcagcaaagtaggaaggttccttacacgttcggaggggggaccaagctggaaataaaacgagggggcggaggatccggtggaggcggaagcgggggtggaggatcccaggtgcagctgcaggagtcaggacctggcctggtgacgccctcacagagcctgtccatcacttgtactgtctctgggttttcattaagcgactatggtgttcattgggttcgccagtctccaggacagggactggagtggctgggagtaatatgggctggtggaggcacgaattataattcggctctcatgtccagaaagagcatcagcaaagacaactccaagagccaagttttcttaaaaatgaacagtctgcaagctgatgacacagccgtgtattactgtgccagagataagggatactcctattactattctatggactactggggccaaggcaccacggtcaccgtctcctcaggaggcggcggcagcggcgggggagggtccggagggggtggttctggtggaggaggatcgggaggcggtggcagccaggtccagctgcagcagtctggggctgaactggcaagacctggggcctcagtgaagatgtcctgcaaggcttctggctacacctttactaggtacacgatgcactgggtaaaacagaggcctggacagggtctggaatggattggatacattaatcctagccgtggttatactaattacaatcagaagttcaaggacaaggccacattgactacagacaaatcctccagcacagcctacatgcaactgagcagcctgacatctgaggactctgcagtctattactgtgcaagatattatgatgatcattactgccttgactactggggccaaggcaccactctcacagtctcctcaggtggcggtggctccggcggtggtgggtcgggtggcggcggatctcagattgtgttgacccagtctccagcaatcatgtctgcatctccaggggagaaggttaccatgacctgcagtgccagctcaagtgtaagttacatgaactggtaccagcagaagtcaggcacctcccccaaaagatggatttatgacacatccaaactggcttctggagtccctgctcacttcaggggcagtgggtctgggacctcttactctctcacaatcagcggcatggaggctgaagatgctgccacttattactgccagcagtggagtagtaacccattcacgttcggctcggggaccaagctggagatcaaccgtgcggccgcaactaccaccttcgaacatcctcacattcaagacgctgcttcgcaacttcctgatgatgagagtttattttttggtgatactgggctatccaaaaatccaatcgagcttgtagaaggttggttcagtagttggaaaagctctattgcctcttttttctttatcatagggttaatcattggactattcttggttctccgagttggtatccatctttgcattaaattaaagcacaccaagaaaagacagatttatacagacatagagatgaaccgacttggaaag

SEQ ID NO: 35 - DNA, 1485 bp, synthetic construct
  source 1..1485: mol_type = other DNA
aagttcaccatagtttttccacacaaccaaaaaggaaactggaaaaatgttccttctaattaccattattgcccgtcaagctcagatttaaattggcataatgacttaataggcacagccttacaagtcaaaatgcccaagagtcacaaggctattcaagcagacggttggatgtgtcatgcttccaaatgggtcactacttgtgatttccgctggtatggaccgaagtatataacacattccatccgatccttcactccatctgtagaacaatgcaaggaaagcattgaacaaacgaaacaaggaacttggctgaatccaggcttccctcctcaaagttgtggatatgcaactgtgacggatgccgaagcagtgattgtccaggtgactcctcaccatgtgctggttgatgaatacacaggagaatgggttgattcacagttcatcaacggaaaatgcagcaattacatatgccccactgtccataactctacaacctggcattctgactataaggtcaaagggctatgtgattctaacctcatttccatggacatcaccttcttctcagaggacggagagctatcatccctgggaaaggagggcacagggttcagaagtaactactttgcttatgaaactggaggcaaggcctgcaaaatgcaatactgcaagcattggggagtcagactcccatcaggtgtctggttcgagatggctgataaggatctctttgctgcagccagattccctgaatgcccagaagggtcaagtatctctgctccatctcagacctcagtggatgtaagtctaattcaggacgttgagaggatcttggattattccctctgccaagaaacctggagcaaaatcagagcgggtcttccaatctctccagtggatctcagctatcttgctcctaaaaacccaggaaccggtcctgctttcaccataatcaatggtaccctaaaatactttgagaccagatacatcagagtcgatattgctgctccaatcctctcaagaatggtcggaatgatcagtggaactaccacagaaagggaactgtgggatgactgggcaccatatgaagacgtggaaattggacccaatggagttctgaggaccagttcaggatataagtttcctttatacatgattggacatggtatgttggactccgatcttcatcttagctcaaaggctcaggtgttcgaacatcctcacattcaagacgctgcttcgcaacttcctgatgatgagagtttattttttggtgatactgggctatccaaaaatccaatcgagcttgtagaaggttggttcagtagttggaaaagctctattgcctcttttttctttatcatagggttaatcattggactattcttggttctccgagttggtatccatctttgcattaaattaaagcacaccaagaaaagacagatttatacagacatagagatgaaccgacttggaaag

SEQ ID NO: 36 - protein, 41 aa, synthetic construct
IIGLIIGLFLVLRVGIHLCIKLKHTKKRQIYTDIEMNRLGK

SEQ ID NO: 37 - protein, 51 aa, synthetic construct
WKSSIASFFFIIGLIIGLFLVLRVGIHLCIKLKHTKKRQIYTDIEMNRLGK

SEQ ID NO: 38 - protein, 61 aa, synthetic construct
IELVEGWFSSWKSSIASFFFIIGLIIGLFLVLRVGIHLCIKLKHTKKRQIYTDIEMNRLGK

SEQ ID NO: 39 - protein, 71 aa, synthetic construct
FGDTGLSKNPIELVEGWFSSWKSSIASFFFIIGLIIGLFLVLRVGIHLCIKLKHTKKRQIYTDIEMNRLGK

SEQ ID NO: 40 - protein, 81 aa, synthetic construct
SQLPDDESLFFGDTGLSKNPIELVEGWFSSWKSSIASFFFIIGLIIGLFLVLRVGIHLCIKLKHTKKRQIYTDIEMNRLGK

SEQ ID NO: 41 - protein, 101 aa, synthetic construct
DLHLSSKAQVFEHPHIQDAASQLPDDESLFFGDTGLSKNPIELVEGWFSSWKSSIASFFFIIGLIIGLFLVLRVGIHLCIKLKHTKKRQIYTDIEMNRLGK

SEQ ID NO: 42 - protein, 111 aa, synthetic construct
YMIGHGMLDSDLHLSSKAQVFEHPHIQDAASQLPDDESLFFGDTGLSKNPIELVEGWFSSWKSSIASFFFIIGLIIGLFLVLRVGIHLCIKLKHTKKRQIYTDIEMNRLGK

SEQ ID NO: 43 - protein, 121 aa, synthetic construct
RTSSGYKFPLYMIGHGMLDSDLHLSSKAQVFEHPHIQDAASQLPDDESLFFGDTGLSKNPIELVEGWFSSWKSSIASFFFIIGLIIGLFLVLRVGIHLCIKLKHTKKRQIYTDIEMNRLGK

SEQ ID NO: 44 - protein, 131 aa, synthetic construct
DVEIGPNGVLRTSSGYKFPLYMIGHGMLDSDLHLSSKAQVFEHPHIQDAASQLPDDESLFFGDTGLSKNPIELVEGWFSSWKSSIASFFFIIGLIIGLFLVLRVGIHLCIKLKHTKKRQIYTDIEMNRLGK

SEQ ID NO: 45 - protein, 141 aa, synthetic construct
ELWDDWAPYEDVEIGPNGVLRTSSGYKFPLYMIGHGMLDSDLHLSSKAQVFEHPHIQDAASQLPDDESLFFGDTGLSKNPIELVEGWFSSWKSSIASFFFIIGLIIGLFLVLRVGIHLCIKLKHTKKRQIYTDIEMNRLGK

SEQ ID NO: 46 - protein, 290 aa, synthetic construct
DIKLQQSGAELARPGASVKMSCKTSGYTFTRYTMHWVKQRPGQGLEWIGYINPSRGYTNYNQKFKDKATLTTDKSSSTAYMQLSSLTSEDSAVYYCARYYDDHYCLDYWGQGTTLTVSSVEGGSGGSGGSGGSGGVDDIQLTQSPAIMSASPGEKVTMTCRASSSVSYMNWYQQKSGTSPKRWIYDTSKVASGVPYRFSGSGSGTSYSLTISSMEAEDAATYYCQQWSSNPLTFGAGTKLELKAAATTTIIGLIIGLFLVLRVGIHLCIKLKHTKKRQIYTDIEMNRLGK

SEQ ID NO: 47 - protein, 300 aa, synthetic construct
DIKLQQSGAELARPGASVKMSCKTSGYTFTRYTMHWVKQRPGQGLEWIGYINPSRGYTNYNQKFKDKATLTTDKSSSTAYMQLSSLTSEDSAVYYCARYYDDHYCLDYWGQGTTLTVSSVEGGSGGSGGSGGSGGVDDIQLTQSPAIMSASPGEKVTMTCRASSSVSYMNWYQQKSGTSPKRWIYDTSKVASGVPYRFSGSGSGTSYSLTISSMEAEDAATYYCQQWSSNPLTFGAGTKLELKAAATTTWKSSIASFFFIIGLIIGLFLVLRVGIHLCIKLKHTKKRQIYTDIEMNRLGK

SEQ ID NO: 48 - protein, 310 aa, synthetic construct
DIKLQQSGAELARPGASVKMSCKTSGYTFTRYTMHWVKQRPGQGLEWIGYINPSRGYTNYNQKFKDKATLTTDKSSSTAYMQLSSLTSEDSAVYYCARYYDDHYCLDYWGQGTTLTVSSVEGGSGGSGGSGGSGGVDDIQLTQSPAIMSASPGEKVTMTCRASSSVSYMNWYQQKSGTSPKRWIYDTSKVASGVPYRFSGSGSGTSYSLTISSMEAEDAATYYCQQWSSNPLTFGAGTKLELKAAATTTIELVEGWFSSWKSSIASFFFIIGLIIGLFLVLRVGIHLCIKLKHTKKRQIYTDIEMNRLGK

SEQ ID NO: 49 - protein, 320 aa, synthetic construct
DIKLQQSGAELARPGASVKMSCKTSGYTFTRYTMHWVKQRPGQGLEWIGYINPSRGYTNYNQKFKDKATLTTDKSSSTAYMQLSSLTSEDSAVYYCARYYDDHYCLDYWGQGTTLTVSSVEGGSGGSGGSGGSGGVDDIQLTQSPAIMSASPGEKVTMTCRASSSVSYMNWYQQKSGTSPKRWIYDTSKVASGVPYRFSGSGSGTSYSLTISSMEAEDAATYYCQQWSSNPLTFGAGTKLELKAAATTTFGDTGLSKNPIELVEGWFSSWKSSIASFFFIIGLIIGLFLVLRVGIHLCIKLKHTKKRQIYTDIEMNRLGK

SEQ ID NO: 50 - protein, 330 aa, synthetic construct
DIKLQQSGAELARPGASVKMSCKTSGYTFTRYTMHWVKQRPGQGLEWIGYINPSRGYTNYNQKFKDKATLTTDKSSSTAYMQLSSLTSEDSAVYYCARYYDDHYCLDYWGQGTTLTVSSVEGGSGGSGGSGGSGGVDDIQLTQSPAIMSASPGEKVTMTCRASSSVSYMNWYQQKSGTSPKRWIYDTSKVASGVPYRFSGSGSGTSYSLTISSMEAEDAATYYCQQWSSNPLTFGAGTKLELKAAATTTSQLPDDESLFFGDTGLSKNPIELVEGWFSSWKSSIASFFFIIGLIIGLFLVLRVGIHLCIKLKHTKKRQIYTDIEMNRLGK

SEQ ID NO: 51 - protein, 350 aa, synthetic construct
DIKLQQSGAELARPGASVKMSCKTSGYTFTRYTMHWVKQRPGQGLEWIGYINPSRGYTNYNQKFKDKATLTTDKSSSTAYMQLSSLTSEDSAVYYCARYYDDHYCLDYWGQGTTLTVSSVEGGSGGSGGSGGSGGVDDIQLTQSPAIMSASPGEKVTMTCRASSSVSYMNWYQQKSGTSPKRWIYDTSKVASGVPYRFSGSGSGTSYSLTISSMEAEDAATYYCQQWSSNPLTFGAGTKLELKAAATTTDLHLSSKAQVFEHPHIQDAASQLPDDESLFFGDTGLSKNPIELVEGWFSSWKSSIASFFFIIGLIIGLFLVLRVGIHLCIKLKHTKKRQIYTDIEMNRLGK

SEQ ID NO: 52 - protein, 360 aa, synthetic construct
DIKLQQSGAELARPGASVKMSCKTSGYTFTRYTMHWVKQRPGQGLEWIGYINPSRGYTNYNQKFKDKATLTTDKSSSTAYMQLSSLTSEDSAVYYCARYYDDHYCLDYWGQGTTLTVSSVEGGSGGSGGSGGSGGVDDIQLTQSPAIMSASPGEKVTMTCRASSSVSYMNWYQQKSGTSPKRWIYDTSKVASGVPYRFSGSGSGTSYSLTISSMEAEDAATYYCQQWSSNPLTFGAGTKLELKAAATTTYMIGHGMLDSDLHLSSKAQVFEHPHIQDAASQLPDDESLFFGDTGLSKNPIELVEGWFSSWKSSIASFFFIIGLIIGLFLVLRVGIHLCIKLKHTKKRQIYTDIEMNRLGK

SEQ ID NO: 53 - protein, 370 aa, synthetic construct
DIKLQQSGAELARPGASVKMSCKTSGYTFTRYTMHWVKQRPGQGLEWIGYINPSRGYTNYNQKFKDKATLTTDKSSSTAYMQLSSLTSEDSAVYYCARYYDDHYCLDYWGQGTTLTVSSVEGGSGGSGGSGGSGGVDDIQLTQSPAIMSASPGEKVTMTCRASSSVSYMNWYQQKSGTSPKRWIYDTSKVASGVPYRFSGSGSGTSYSLTISSMEAEDAATYYCQQWSSNPLTFGAGTKLELKAAATTTRTSSGYKFPLYMIGHGMLDSDLHLSSKAQVFEHPHIQDAASQLPDDESLFFGDTGLSKNPIELVEGWFSSWKSSIASFFFIIGLIIGLFLVLRVGIHLCIKLKHTKKRQIYTDIEMNRLGK

SEQ ID NO: 54 - protein, 380 aa, synthetic construct
DIKLQQSGAELARPGASVKMSCKTSGYTFTRYTMHWVKQRPGQGLEWIGYINPSRGYTNYNQKFKDKATLTTDKSSSTAYMQLSSLTSEDSAVYYCARYYDDHYCLDYWGQGTTLTVSSVEGGSGGSGGSGGSGGVDDIQLTQSPAIMSASPGEKVTMTCRASSSVSYMNWYQQKSGTSPKRWIYDTSKVASGVPYRFSGSGSGTSYSLTISSMEAEDAATYYCQQWSSNPLTFGAGTKLELKAAATTTDVEIGPNGVLRTSSGYKFPLYMIGHGMLDSDLHLSSKAQVFEHPHIQDAASQLPDDESLFFGDTGLSKNPIELVEGWFSSWKSSIASFFFIIGLIIGLFLVLRVGIHLCIKLKHTKKRQIYTDIEMNRLGK

SEQ ID NO: 55 - protein, 390 aa, synthetic construct
DIKLQQSGAELARPGASVKMSCKTSGYTFTRYTMHWVKQRPGQGLEWIGYINPSRGYTNYNQKFKDKATLTTDKSSSTAYMQLSSLTSEDSAVYYCARYYDDHYCLDYWGQGTTLTVSSVEGGSGGSGGSGGSGGVDDIQLTQSPAIMSASPGEKVTMTCRASSSVSYMNWYQQKSGTSPKRWIYDTSKVASGVPYRFSGSGSGTSYSLTISSMEAEDAATYYCQQWSSNPLTFGAGTKLELKAAATTTELWDDWAPYEDVEIGPNGVLRTSSGYKFPLYMIGHGMLDSDLHLSSKAQVFEHPHIQDAASQLPDDESLFFGDTGLSKNPIELVEGWFSSWKSSIASFFFIIGLIIGLFLVLRVGIHLCIKLKHTKKRQIYTDIEMNRLGK

SEQ ID NO: 56 - protein, 744 aa, synthetic construct
DIKLQQSGAELARPGASVKMSCKTSGYTFTRYTMHWVKQRPGQGLEWIGYINPSRGYTNYNQKFKDKATLTTDKSSSTAYMQLSSLTSEDSAVYYCARYYDDHYCLDYWGQGTTLTVSSVEGGSGGSGGSGGSGGVDDIQLTQSPAIMSASPGEKVTMTCRASSSVSYMNWYQQKSGTSPKRWIYDTSKVASGVPYRFSGSGSGTSYSLTISSMEAEDAATYYCQQWSSNPLTFGAGTKLELKAAATTTKFTIVFPHNQKGNWKNVPSNYHYCPSSSDLNWHNDLIGTALQVKMPKSHKAIQADGWMCHASKWVTTCDFRWYGPKYITHSIRSFTPSVEQCKESIEQTKQGTWLNPGFPPQSCGYATVTDAEAVIVQVTPHHVLVDEYTGEWVDSQFINGKCSNYICPTVHNSTTWHSDYKVKGLCDSNLISMDITFFSEDGELSSLGKEGTGFRSNYFAYETGGKACKMQYCKHWGVRLPSGVWFEMADKDLFAAARFPECPEGSSISAPSQTSVDVSLIQDVERILDYSLCQETWSKIRAGLPISPVDLSYLAPKNPGTGPAFTIINGTLKYFETRYIRVDIAAPILSRMVGMISGTTTERELWDDWAPYEDVEIGPNGVLRTSSGYKFPLYMIGHGMLDSDLHLSSKAQVFEHPHIQDAASQLPDDESLFFGDTGLSKNPIELVEGWFSSWKSSIASFFFIIGLIIGLFLVLRVGIHLCIKLKHTKKRQIYTDIEMNRLGK